European Patent Application EP 4 681 733 A2, published January 21, 2026. Title: ANTI-CERAMIDE ANTIBODIES. Applicant: MEMORIAL SLOAN-KETTERING CANCER CENTER. Application US 17/887,952, filed August 15, 2022. The sequence listing filed with the application follows.

SEQUENCE LISTING (51 sequences)

SEQ ID NO: 1 - protein, 10 aa, synthetic construct
  source 1..10: note = Description of Artificial Sequence: Synthetic heavy chain variable region CDR1 of the anti-ceramide antibody
GYTFTDHTIH

SEQ ID NO: 2 - protein, 17 aa, synthetic construct
  source 1..17: note = Description of Artificial Sequence: Synthetic heavy chain variable region CDR2
YNYPRDGSTKYNEKFKG

SEQ ID NO: 3 - protein, 11 aa, synthetic construct
  source 1..11: note = Description of Artificial Sequence: Synthetic heavy chain variable region CDR3
GFITTVVPSAY

SEQ ID NO: 4 - protein, 11 aa, synthetic construct
  source 1..11: note = Description of Artificial Sequence: Synthetic light chain variable region CDR1
RASKSISKYLA

SEQ ID NO: 5 - protein, 7 aa, synthetic construct
  source 1..7: note = Description of Artificial Sequence: Synthetic light chain variable region CDR2
SGSTLQS

SEQ ID NO: 6 - protein, 9 aa, synthetic construct
  source 1..9: note = Description of Artificial Sequence: Synthetic light chain variable region CDR3
QQHNEYPWT

SEQ ID NO: 7 - protein, 119 aa, synthetic construct
  source 1..119: note = Description of Artificial Sequence: Synthetic heavy chain variable region sequence
QVQLQQSDAELVKPGASVKISCKVSGYTFTDHTIHWMKQRPEQGLEWIGYNPRDGSTKYNEKFGKATLTDADKSSSTAYMQLNSLTSEDSAVYFCAKGFITTVVPSAYWGQGTLVTVSA

SEQ ID NO: 8 - protein, 107 aa, synthetic construct
  source 1..107: note = Description of Artificial Sequence: Synthetic light chain variable region sequence
DVQITQSPSYLAASPGETITINCRASKSISKYLAWYQEKPGKTNKLLIYSGSTLQSGIPSRFSGSGSGTDFTLTISSLEPEDFAMYYCQQHNEYPWTFGGGTKLEIK

SEQ ID NO: 9 - protein, 10 aa, synthetic construct
  source 1..10: note = Description of Artificial Sequence: Synthetic heavy chain variable region CDR1
GYAFSSYWMN

SEQ ID NO: 10 - protein, 17 aa, synthetic construct
  source 1..17: note = Description of Artificial Sequence: Synthetic heavy chain variable region CDR2
QIYPGDGDTNYNGKFKG

SEQ ID NO: 11 - protein, 10 aa, synthetic construct
  source 1..10: note = Description of Artificial Sequence: Synthetic heavy chain variable region CDR3
RCYYGLYFDV

SEQ ID NO: 12 - protein, 11 aa, synthetic construct
  source 1..11: note = Description of Artificial Sequence: Synthetic light chain variable region CDR1
KASQDINRYLS

SEQ ID NO: 13 - protein, 7 aa, synthetic construct
  source 1..7: note = Description of Artificial Sequence: Synthetic light chain variable region CDR2
RANRLVD

SEQ ID NO: 14 - protein, 9 aa, synthetic construct
  source 1..9: note = Description of Artificial Sequence: Synthetic light chain variable region CDR3
LQYDEFPYT

SEQ ID NO: 15 - protein, 119 aa, synthetic construct
  source 1..119: note = Description of Artificial Sequence: Synthetic heavy chain variable region sequence
QVQLQQSGAELVKPGASVKISCKASGYAFSSYWMNWVKQRPGKGLEWIGQIYPGDGDTNYNGKFKGKATLTADKSSSTAYMQLSSLTSEDSAVYFCTRRCYYGLYFDVWGTGTTVTVSS

SEQ ID NO: 16 - protein, 108 aa, synthetic construct
  source 1..108: note = Description of Artificial Sequence: Synthetic light chain variable region sequence
DIKMTQSPSSRYASLGERVTITCKASQDINRYLSWFQQKPGKSPKTLIYRANRLVDGVPSSRFSGSGSGQDYSLTISSLEYEDMGIYYCLQYDEFPYTFGGGTKLEIK

SEQ ID NO: 17 - protein, 10 aa, synthetic construct
  source 1..10: note = Description of Artificial Sequence: Synthetic heavy chain variable region CDR1 of the anti-ceramide antibody
GYTFTSYWMH

SEQ ID NO: 18 - protein, 16 aa, synthetic construct
  source 1..16: note = Description of Artificial Sequence: Synthetic heavy chain variable region CDR2
YINPSSGYTKYNQFKD

SEQ ID NO: 19 - protein, 8 aa, synthetic construct
  source 1..8: note = Description of Artificial Sequence: Synthetic heavy chain variable region CDR3
GGYYGFAY

SEQ ID NO: 20 - protein, 10 aa, synthetic construct
  source 1..10: note = Description of Artificial Sequence: Synthetic light chain variable region CDR1
SASSSVSYMY

SEQ ID NO: 21 - protein, 7 aa, synthetic construct
  source 1..7: note = Description of Artificial Sequence: Synthetic light chain variable region CDR2
LTSNLAS

SEQ ID NO: 22 - protein, 9 aa, synthetic construct
  source 1..9: note = Description of Artificial Sequence: Synthetic light chain variable region CDR3
QQWSSNPLT

SEQ ID NO: 23 - protein, 117 aa, synthetic construct
  source 1..117: note = Description of Artificial Sequence: Synthetic heavy chain variable region sequence
QVQLQQSGAELAKPGASVKLSCKASGYTFTSYWMHWVKQRPGQGLEWIGYINPSSGYTKYNQKFKDKATLTADKSSSTAYMQLSSLTYEDSAVYYCARGGYYGFAYWGQGTLVTVSA

SEQ ID NO: 24 - protein, 106 aa, synthetic construct
  source 1..106: note = Description of Artificial Sequence: Synthetic light chain variable region sequence
QIVLTQSPALMSASPGEKVTMTCSASSSVSYMYWYQQKPRSSPKPWIYLTSNLASGVPARFSGSGSGTSYSLTISSMEAEDAATYYCQQWSSNPLTFGAGTKLELK

SEQ ID NO: 25 - protein, 10 aa, synthetic construct
  source 1..10: note = Description of Artificial Sequence: Synthetic heavy chain variable region CDR1 of the anti-ceramide antibody
GFSLTGYGVH

SEQ ID NO: 26 - protein, 16 aa, synthetic construct
  source 1..16: note = Description of Artificial Sequence: Synthetic heavy chain variable region CDR2
VIWSGGSTDYNAAFIS

SEQ ID NO: 27 - protein, 10 aa, synthetic construct
  source 1..10: note = Description of Artificial Sequence: Synthetic heavy chain variable region CDR3
NYGYDYAMDY

SEQ ID NO: 28 - protein, 11 aa, synthetic construct
  source 1..11: note = Description of Artificial Sequence: Synthetic light chain variable region CDR1
RASQSIGTSIH

SEQ ID NO: 29 - protein, 7 aa, synthetic construct
  source 1..7: note = Description of Artificial Sequence: Synthetic light chain variable region CDR2
YASESIS

SEQ ID NO: 30 - protein, 9 aa, synthetic construct
  source 1..9: note = Description of Artificial Sequence: Synthetic light chain variable region CDR3
QQSNSWPFT

SEQ ID NO: 31 - protein, 116 aa, synthetic construct
  source 1..116: note = Description of Artificial Sequence: Synthetic heavy chain variable region sequence
QVQLKQSGPGVQPSSLSITCTVSGFSLTSYGVHWVRQSPGKGLEWLGVIWSGGSTDYNAAFISRLSISKDNSKSQVFFKMNSLQADDTAIYYCARNYGYDYAMDYWGQGTSVTVSS

SEQ ID NO: 32 - protein, 107 aa, synthetic construct
  source 1..107: note = Description of Artificial Sequence: Synthetic light chain variable region sequence
DILLTQSPAILSVSPGERVSFSCRASQSIGTSIHWYQQRTNGSPRLLIKYASESISGIPSRFSGSGSGTDFTLSINSVESEDIADYYCQQSNSWPFTFGSGTKLEIK

SEQ ID NO: 33 - protein, 10 aa, synthetic construct
  source 1..10: note = Description of Artificial Sequence: Synthetic heavy chain variable region CDR1 of the anti-ceramide antibody
GYTFTNYWMH

SEQ ID NO: 34 - protein, 17 aa, synthetic construct
  source 1..17: note = Description of Artificial Sequence: Synthetic heavy chain variable region CDR2
AIYPGDSDTSYNQKFKG

SEQ ID NO: 35 - protein, 7 aa, synthetic construct
  source 1..7: note = Description of Artificial Sequence: Synthetic heavy chain variable region CDR3
GLYYGYD

SEQ ID NO: 36 - protein, 16 aa, synthetic construct
  source 1..16: note = Description of Artificial Sequence: Synthetic light chain variable region CDR1
KSSQSLIDSDGKTFLN

SEQ ID NO: 37 - protein, 7 aa, synthetic construct
  source 1..7: note = Description of Artificial Sequence: Synthetic light chain variable region CDR2
LVSKLDS

SEQ ID NO: 38 - protein, 9 aa, synthetic construct
  source 1..9: note = Description of Artificial Sequence: Synthetic said light chain variable region CDR3
WQGTHFPYT

SEQ ID NO: 39 - protein, 115 aa, synthetic construct
  source 1..115: note = Description of Artificial Sequence: Synthetic heavy chain variable region sequence comprising the sequence
EVQLQQSGTVLARPGASVKMSCKASGYTFTNYWMHWVKQRPVQGLEWIGAIYPGDSDTSYNQKFKGKAKLTAVTSTSTAFMELSSLTNEDSAVYYCTGLYYGYDWGQGTTLTVSS

SEQ ID NO: 40 - protein, 112 aa, synthetic construct
  source 1..112: note = Description of Artificial Sequence: Synthetic light chain variable region sequence
DVLMTQTPLTLSVTIGQPASISCKSSQSLIDSDGKTFLNWLLQRPGQSPKRLIYLVSKLDSGVPDRFTGSGSGTDFTLKISRVEAEDLGLYYCWQGTHFPYTFGGGTKLEIK

SEQ ID NO: 41 - protein, 109 aa, Homo sapiens
  source 1..109: note = Human V gene 1-46
QVQLVQSGAEVKKPGASVKVSCKASGYTFTSYYMHWVRQAPGQGLEWMGIINPSGGSTSYAQKFQGRVTMTRDTSTSTVYMELSSLRSEDTAVYYCARWGQGTTVTVSS

SEQ ID NO: 42 - protein, 113 aa, synthetic construct
  source 1..113: note = Description of Artificial Sequence: Synthetic VL 2A2
DVLMTQTPLTLSVTIGQPASISCKSSQSLIDSDGKTFLNWLLQRPGQSPKRLIYLVSKLDSGVPDRFTGSGSGTDFTLKISRVEAEDLGLYYCWQGTHFPYTFGGGTKLEIKR

SEQ ID NO: 43 - protein, 112 aa, Homo sapiens
  source 1..112: note = Human V gene A1
DVVMTQSPLSLPVTLGQPASISCRSSQSLVYSDGNTYLNWFQQRPGQSPRRLIYKVSNWDSGVPDRFSGSGSGTDFTLKISRVEAEDVGVYYCMQGTHWPTFGQGTKLEIKR

SEQ ID NO: 44 - DNA, 1395 bp, synthetic construct
  source 1..1395: mol_type = other DNA; note = Description of Artificial Sequence: Synthetic Humanized 2A2 Heavy chain sequence
atggactggacctggagggtcttctgcttgctggctgtagctccaggtgctcactcccaggtgcagcttgtgcagtctggggctgaggtgaaaaagcctggggcttcagtgaaggtgtcctgcaaggcttctggctacacctttaccaactactggatgcactgggtaagacaggcgcctggacagggtctggaatggatgggcgctatttatcctggagatagtgatactagctacaaccagaagttcaagggccgggtcacaatgactcgagacacatccaccagcactgtctacatggagctcagcagcctgagaagtgaggacactgcggtctattactgtgcacgcctttactacggctacgactggggccaaggcaccactgtcacagtctcctcagccagcacgaagggcccatcggtcttccccctggcaccctcctccaagagcacctctgggggcacagcggccctgggctgcctggtcaaggactacttccccgaaccggtgacggtgtcgtggaactcaggcgccctgaccagcggcgtgcacaccttcccggctgtcctacagtcctcaggactctactccctcagcagcgtggtgaccgtgccctccagcagcttgggcacccagacctacatctgcaacgtgaatcacaagcccagcaacaccaaggtggacaagaaagttgagcccaaatcttgtgacaaaactcacacatgcccaccgtgcccagcacctgaactcctggggggaccgtcagtcttcctcttccccccaaaacccaaggacaccctcatgatctcccggacccctgaggtcacatgcgtggtggtggacgtgagccacgaagaccctgaggtcaagttcaactggtacgtggacggcgtggaggtgcataatgccaagacaaagccgcgggaggagcagtacaacagcacgtaccgtgtggtcagcgtcctcaccgtcctgcaccaggactggctgaatggcaaggagtacaagtgcaaggtctccaacaaagccctcccagcccccatcgagaaaaccatctccaaagccaaagggcagccccgagaaccacaggtgtacaccctgcccccatcccgggatgagctgaccaagaaccaggtcagcctgacctgcctggtcaaaggcttctatcccagcgacatcgccgtggagtgggagagcaatgggcagccggagaacaactacaagaccacgcctcccgtgctggactccgacggctccttcttcctctacagcaagctcaccgtggacaagagcaggtggcagcaggggaacgtcttctcatgctccgtgatgcatgaggctctgcacaaccactacacgcagaagagcctctccctgtccccgggtaaatga

SEQ ID NO: 45 - protein, 463 aa, synthetic construct
  source 1..463: note = Description of Artificial Sequence: Synthetic Humanized 2A2 Heavy chain sequence
MDWTWRVFCLLAVAPGAHSQVQLVQSGAEVKKPGASVKVSCKASGYTFTNYWMHWVRQAPGQGLEWMGAIYPGDSDTSYNQKFKGRVTMTRDTSTSTVYMELSSLRSEDTAVYYCARLYYGYDWGQGTTVTVSSASTKGPSVFPLAPSSKSTSGGTAALGCLVKDYFPEPVTVSWNSGALTSGVHTFPAVLQSSGLYSLSSVVTVPSSSLGTQTYICNVNHKPSNTKVDKKVEPKSCDKTHTCPPCPAPELLGGPSVFLFPPKPKDTLMISRTPEVTCVVVDVSHEDPEVKFNWYVDGVEVHNAKTKPREEQYNSTYRVVSVLTVLHQDWLNGKEYKCKVSNKALPAPIEKTISKAKGQPREPQVYTLPPSRDELTKNQVSLTCLVKGFYPSDIAVEWESNGQPENNYKTTPPVLDSDGSFFLYSKLTVDKSRWQQGNVFSCSVMHEALHNHYTQKSLSLSPG

SEQ ID NO: 46 - DNA, 720 bp, synthetic construct
  source 1..720: mol_type = other DNA; note = Description of Artificial Sequence: Synthetic polynucleotide
atgaggctccctgctcagctcctggggctgctaatgctctgggtcccaggatccagtggggatgttgtgatgacccaatctccactctctttgccggttacccttggacaaccagcctccatctcttgcaagtcaagtcagagcctcatagatagtgatggaaagacatttttgaattggttccaacagaggccaggccagtctccaaggcgcctaatctatctggtgtctaaactggactctggagtccctgacaggttctctggcagtggatcagggacagatttcactctgaaaatcagcagagtggaggctgaggatgtgggagtttattattgctggcaaggtacacattttccgtacacgttcggacaggggaccaagctggaaataaaacggacggtggctgcaccatctgtcttcatcttcccgccatctgatgagcagttgaaatctggaactgcctctgttgtgtgcctgctgaataacttctatcccagagaggccaaagtacagtggaaggtggataacgccctccaatcgggtaactcccaggagagtgtcacagagcaggacagcaaggacagcacctacagcctcagcagcaccctgacgctgagcaaagcagactacgagaaacacaaagtctacgcctgcgaagtcacccatcagggcctgagttcgcccgtcacaaagagcttcaacaggggagagtgttaa

SEQ ID NO: 47 - protein, 239 aa, synthetic construct
  source 1..239: note = Description of Artificial Sequence: Synthetic polypeptide
MRLPAQLLGLLMLWVPGSSGDVVMTQSPLSLPVTLGQPASISCKSSQSLIDSDGKTFLNWFQQRPGQSPRRLIYLVSKLDSGVPDRFSGSGSGTDFTLKISRVEAEDVGVYYCWQGTHFPYTFGQGTKLEIKRTVAAPSVFIFPPSDEQLKSGTASVVCLLNNFYPREAKVQWKVDNALQSGNSQESVTEQDSKDSTYSLSSTLTLSKADYEKHKVYACEVTHQGLSSPVTKSFNRGEC

SEQ ID NO: 48 - protein, 120 aa, synthetic construct
  source 1..120: note = Description of Artificial Sequence: Synthetic polypeptide
QVQLQQSDAELVKPGASVKISCKVSGYTFTDHTIHWMKQRPEQGLEWIGYNYPRDGSTKYNEKFKGKATLTADKSSSTAYMQLNSLTSEDSAVYFCAKGFITTVVPSAYWGQGTLVTVSA

SEQ ID NO: 49 - protein, 118 aa, synthetic construct
  source 1..118: note = Description of Artificial Sequence: Synthetic polypeptide
QVQLKQSGPGLVQPSQSLSITCTVSGFSLTSYGVHWVRQSPGKGLEWLGVIWSGGSTDYNAAFISRLSISKDNSKSQVFFKMNSLQADDTAIYYCARNYGYDYAMDYWGQGTSVTVSS

SEQ ID NO: 50 - protein, 115 aa, synthetic construct
  source 1..115: note = Description of Artificial Sequence: Synthetic polypeptide
QVQLVQSGAEVKKPGASVKVSCKASGYTFTNYWMHWVRQAPGQGLEWMGAIYPGDSDTSYNQKFKGRVTMTRDTSTSTVYMELSSLRSEDTAVYYCARLYYGYDWGQGTTVTVSS

SEQ ID NO: 51 - protein, 107 aa, synthetic construct
  source 1..107: note = Description of Artificial Sequence: Synthetic polypeptide
DIKMTQSPSSRYASLGERVTITCKASQDINRYLSWFQQKPGKSPKTLIYRANRLVDGVPSRFSGSGSGQDYSLTISSLEYEDMGIYYCLQYDEFPYTFGGGTKLEIK